European Patent Application EP 4 512 898 A1, published February 26, 2025. Title: 一种封闭序列及其试剂盒和使用方法. Applicant: 京东方科技集团股份有限公司. The sequence listing filed with the application follows.

SEQUENCE LISTING (43 sequences)

SEQ ID NO: 1 - DNA, 28 bp, synthetic construct
  source 1..28: mol_type = other DNA
tgtagatctcggtggtcgccgtatcatt

SEQ ID NO: 2 - DNA, 33 bp, synthetic construct
  source 1..33: mol_type = other DNA
agatcggaagagcgtcgtgtagggaaagagtgt

SEQ ID NO: 3 - DNA, 27 bp, synthetic construct
  source 1..27: mol_type = other DNA
aagagcacacgtctgaactccagtcac

SEQ ID NO: 4 - DNA, 24 bp, synthetic construct
  source 1..24: mol_type = other DNA
atctcgtatgccgtcttctgcttg

SEQ ID NO: 5 - DNA, 70 bp, synthetic construct
  source 1..70: mol_type = other DNA
aatgatacggcgaccaccgagatctacacaatggtcgacactctttccctacacgacgctcttccgatct

SEQ ID NO: 6 - DNA, 65 bp, synthetic construct
  source 1..65: mol_type = other DNA
gatcggaagagcacacgtctgaactccagtcactgataggcatctcgtatgccgtcttctgcttg

SEQ ID NO: 7 - DNA, 70 bp, synthetic construct
  source 1..70: mol_type = other DNA
aatgatacggcgaccaccgagatctacactcgctatcacactctttccctacacgacgctcttccgatct

SEQ ID NO: 8 - DNA, 65 bp, synthetic construct
  source 1..65: mol_type = other DNA
gatcggaagagcacacgtctgaactccagtcaccatccaagatctcgtatgccgtcttctgcttg

SEQ ID NO: 9 - DNA, 70 bp, synthetic construct
  source 1..70: mol_type = other DNA
aatgatacggcgaccaccgagatctacaccgtccattacactctttccctacacgacgctcttccgatct

SEQ ID NO: 10 - DNA, 65 bp, synthetic construct
  source 1..65: mol_type = other DNA
gatcggaagagcacacgtctgaactccagtcacgtgagactatctcgtatgccgtcttctgcttg

SEQ ID NO: 11 - DNA, 70 bp, synthetic construct
  source 1..70: mol_type = other DNA
aatgatacggcgaccaccgagatctacactactagcgacactctttccctacacgacgctcttccgatct

SEQ ID NO: 12 - DNA, 65 bp, synthetic construct
  source 1..65: mol_type = other DNA
gatcggaagagcacacgtctgaactccagtcacctgatgagatctcgtatgccgtcttctgcttg

SEQ ID NO: 13 - DNA, 70 bp, synthetic construct
  source 1..70: mol_type = other DNA
aatgatacggcgaccaccgagatctacaccctagagaacactctttccctacacgacgctcttccgatct

SEQ ID NO: 14 - DNA, 65 bp, synthetic construct
  source 1..65: mol_type = other DNA
gatcggaagagcacacgtctgaactccagtcacacggtacaatctcgtatgccgtcttctgcttg

SEQ ID NO: 15 - DNA, 70 bp, synthetic construct
  source 1..70: mol_type = other DNA
aatgatacggcgaccaccgagatctacaccgcaatgtacactctttccctacacgacgctcttccgatct

SEQ ID NO: 16 - DNA, 65 bp, synthetic construct
  source 1..65: mol_type = other DNA
gatcggaagagcacacgtctgaactccagtcacctcgacttatctcgtatgccgtcttctgcttg

SEQ ID NO: 17 - DNA, 70 bp, synthetic construct
  source 1..70: mol_type = other DNA
aatgatacggcgaccaccgagatctacacacacctcaacactctttccctacacgacgctcttccgatct

SEQ ID NO: 18 - DNA, 65 bp, synthetic construct
  source 1..65: mol_type = other DNA
gatcggaagagcacacgtctgaactccagtcacacaacgtgatctcgtatgccgtcttctgcttg

SEQ ID NO: 19 - DNA, 70 bp, synthetic construct
  source 1..70: mol_type = other DNA
aatgatacggcgaccaccgagatctacacgaggcattacactctttccctacacgacgctcttccgatct

SEQ ID NO: 20 - DNA, 65 bp, synthetic construct
  source 1..65: mol_type = other DNA
gatcggaagagcacacgtctgaactccagtcactgctgtgaatctcgtatgccgtcttctgcttg

SEQ ID NO: 21 - DNA, 70 bp, synthetic construct
  source 1..70: mol_type = other DNA
aatgatacggcgaccaccgagatctacactactccagacactctttccctacacgacgctcttccgatct

SEQ ID NO: 22 - DNA, 65 bp, synthetic construct
  source 1..65: mol_type = other DNA
gatcggaagagcacacgtctgaactccagtcacccaagtagatctcgtatgccgtcttctgcttg

SEQ ID NO: 23 - DNA, 70 bp, synthetic construct
  source 1..70: mol_type = other DNA
aatgatacggcgaccaccgagatctacaccagcatacacactctttccctacacgacgctcttccgatct

SEQ ID NO: 24 - DNA, 65 bp, synthetic construct
  source 1..65: mol_type = other DNA
gatcggaagagcacacgtctgaactccagtcacaactgaggatctcgtatgccgtcttctgcttg

SEQ ID NO: 25 - DNA, 70 bp, synthetic construct
  source 1..70: mol_type = other DNA
aatgatacggcgaccaccgagatctacacactctccaacactctttccctacacgacgctcttccgatct

SEQ ID NO: 26 - DNA, 65 bp, synthetic construct
  source 1..65: mol_type = other DNA
gatcggaagagcacacgtctgaactccagtcacaggtaggaatctcgtatgccgtcttctgcttg

SEQ ID NO: 27 - DNA, 70 bp, synthetic construct
  source 1..70: mol_type = other DNA
aatgatacggcgaccaccgagatctacacctctatcgacactctttccctacacgacgctcttccgatct

SEQ ID NO: 28 - DNA, 65 bp, synthetic construct
  source 1..65: mol_type = other DNA
gatcggaagagcacacgtctgaactccagtcacttcgccatatctcgtatgccgtcttctgcttg

SEQ ID NO: 29 - DNA, 70 bp, synthetic construct
  source 1..70: mol_type = other DNA
aatgatacggcgaccaccgagatctacacgcaatgagacactctttccctacacgacgctcttccgatct

SEQ ID NO: 30 - DNA, 65 bp, synthetic construct
  source 1..65: mol_type = other DNA
gatcggaagagcacacgtctgaactccagtcaccaggtaagatctcgtatgccgtcttctgcttg

SEQ ID NO: 31 - DNA, 70 bp, synthetic construct
  source 1..70: mol_type = other DNA
aatgatacggcgaccaccgagatctacacaagctggtacactctttccctacacgacgctcttccgatct

SEQ ID NO: 32 - DNA, 65 bp, synthetic construct
  source 1..65: mol_type = other DNA
gatcggaagagcacacgtctgaactccagtcacgtatcgagatctcgtatgccgtcttctgcttg

SEQ ID NO: 33 - DNA, 70 bp, synthetic construct
  source 1..70: mol_type = other DNA
aatgatacggcgaccaccgagatctacaccacgattcacactctttccctacacgacgctcttccgatct

SEQ ID NO: 34 - DNA, 65 bp, synthetic construct
  source 1..65: mol_type = other DNA
gatcggaagagcacacgtctgaactccagtcacttcacggaatctcgtatgccgtcttctgcttg

SEQ ID NO: 35 - DNA, 70 bp, synthetic construct
  source 1..70: mol_type = other DNA
aatgatacggcgaccaccgagatctacacagaagcctacactctttccctacacgacgctcttccgatct

SEQ ID NO: 36 - DNA, 65 bp, synthetic construct
  source 1..65: mol_type = other DNA
gatcggaagagcacacgtctgaactccagtcacgagctctaatctcgtatgccgtcttctgcttg

SEQ ID NO: 37 - DNA, 70 bp, synthetic construct
  source 1..70: mol_type = other DNA
aatgatacggcgaccaccgagatctacacnnnnnnnnacactctttccctacacgacgctcttccgatct

SEQ ID NO: 38 - DNA, 65 bp, synthetic construct
  source 1..65: mol_type = other DNA
gatcggaagagcacacgtctgaactccagtcacnnnnnnnnatctcgtatgccgtcttctgcttg

SEQ ID NO: 39 - DNA, 29 bp, synthetic construct
  source 1..29: mol_type = other DNA
aatgatacggcgaccaccgagatctacac

SEQ ID NO: 40 - DNA, 33 bp, synthetic construct
  source 1..33: mol_type = other DNA
acactctttccctacacgacgctcttccgatct

SEQ ID NO: 41 - DNA, 33 bp, synthetic construct
  source 1..33: mol_type = other DNA
gatcggaagagcacacgtctgaactccagtcac

SEQ ID NO: 42 - DNA, 24 bp, synthetic construct
  source 1..24: mol_type = other DNA
atctcgtatgccgtcttctgcttg

SEQ ID NO: 43 - DNA, 33 bp, synthetic construct; identical to SEQ ID NO: 41
  source 1..33: mol_type = other DNA